European Patent Application EP 4 115 894 A1, published January 11, 2023. Title: Self-Limiting Viral Vectors Encoding Nucleases. Applicant: Precision Biosciences, Inc. The sequence listing filed with the application follows.

SEQUENCE LISTING (10 sequences)

SEQ ID NO: 1 - protein, 163 aa, Chlamydomonas reinhardtii
MNTKYNKEFLLYLAGFVDGDGSIIAQIKPNQSYKFKHQLSLAFQVTQKTQRRWFLDKLVDEIGVGYVRDRGSVSDYILSEIKPLHNFLTQLQPFLKLKQKQANLVLKIIWRLPSAKESPDKFLEVCTWVDQIAALNDSKTRKTTSETVRAVLDSLSEKKKSSP

SEQ ID NO: 2 - DNA, 260 bp, Homo sapiens
gtaagcgcccctaaaatccctttgggcacaatgtgtcctgaggggagaggcagcgacctgtagatgggacgggggcactaaccctcaggtttggggcttctgaatgtgagtatcgccatgtaagcccagtatttggccaatctcagaaagctcctggtccctggagggatggagagagaaaaacaaacagctcctggagcagggagagtgctggcctcttgctctccggctccctctgttgccctctggtttctccccag

SEQ ID NO: 3 - DNA, 346 bp, Polyomavirus SV40
gtatttgcttcttccttaaatcctggtgttgatgcaatgtactgcaaacaatggcctgagtgtgcaaagaaaatgtctgctaactgcatatgcttgctgtgcttactgaggatgaagcatgaaaatagaaaattatacaggaaagatccacttgtgtgggttgattgctactgcttcgattgctttagaatgtggtttggacttgatctttgtgaaggaaccttacttctgtggtgtgacataattggacaaactacctacagagatttaaagctctaaggtaaatataaaatttttaagtgtataatgtgttaaactactgattctaattgtttgtgtattttag

SEQ ID NO: 4 - DNA, 9071 bp, Artificial Sequence
  Synthesized
tcgcgcgtttcggtgatgacggtgaaaacctctgacacatgcagctcccggagacggtcacagcttgtctgtaagcggatgccgggagcagacaagcccgtcagggcgcgtcagcgggtgttggcgggtgtcggggctggcttaactatgcggcatcagagcagattgtactgagagtgcaccatatgcggtgtgaaataccgcacagatgcgtaaggagaaaataccgcatcaggcgccattcgccattcaggctgcgcaactgttgggaagggcgatcggtgcgggcctcttcgctattacgccagctggcgaaagggggatgtgctgcaaggcgattaagttgggtaacgccagggttttcccagtcacgacgttgtaaaacgacggccagtgaattcagatcttcaatattggccattagccatattattcattggttatatagcataaatcaatattggctattggccattgcatacgttgtatctatatcataatatgtacatttatattggctcatgtccaatatgaccgccatgttggcattgattattgactagttattaatagtaatcaattacggggtcattagttcatagcccatatatggagttccgcgttacataacttacggtaaatggcccgcctggctgaccgcccaacgacccccgcccattgacgtcaataatgacgtatgttcccatagtaacgccaatagggactttccattgacgtcaatgggtggagtatttacggtaaactgcccacttggcagtacatcaagtgtatcatatgccaagtccgccccctattgacgtcaatgacggtaaatggcccgcctggcattatgcccagtacatgaccttacgggactttcctacttggcagtacatctacgtattagtcatcgctattaccatgatgatgcggttttggcagtacaccaatgggcgtggatagcggtttgactcacggggatttccaagtctccaccccattgacgtcaatgggagtttgttttggcaccaaaatcaacgggactttccaaaatgtcgtaataaccccgccccgttgacgcaaatgggcggtaggcgtgtacggtgggaggtctatataagcagagctcgtttagtgaaccgtcagatcactagaagcttaattgtgagcgctcacaattgtgagactgctgccgcagtcagtaattgtgagcgctcacaattgacctggagctgcaggagttggtaattgtgagcgctcacaattctcgagatatatatctaggccaccatggcaccgaagaagaagcgcaaggtgcatatgaatacaaaatataataaggtaagtatcaaggttacaagacaggtttaaggcgccaatagaagcttggcttgtcgagacagagaagactcttgcgtttctgataggcacctattggtcttactgacatccactttgcctttctctccacaggagttcttactctacttagcagggtttgtagacggtgacggttccatctttgcctgtatccatcctagtcaagcgtataagttcaagcaccggctgactctccatttcacggtcactcagaagacacagcgccgttggttcctcgacaagctggtggacgagatcggtgtgggttacgtgcaggacgtgggcagcgtctcccagtaccggctgtcccagatcaagcctttgcataattttttaacacaactacaaccttttctaaaactaaaacaaaaacaagcaaatttagttttaaaaattattgaacaacttccgtcagcaaaagaatccccggacaaattcttagaagtttgtacatgggtggatcaaattgcagctctgaatgattcgaagacgcgtaaaacaacttctgaaaccgttcgtgctgtgctagacagtttaccaggatccgtgggaggtctatcgccatctcaggcatccagcgccgcatcctcggcttcctcaagcccgggttcagggatctccgaagcactcagagctggagcaggttccggcactggatacaacaaggaattcctgctctacctggcgggcttcgtcgacggggacggctccatctctgccactatcgctccggctcagtatggtaagttcaagcactatctggggctccggttctatgtcagtcagaagacacagcgccgttggttcctcgacaagctggtggacgagatcggtgtgggttacgtgagtgaccagggcagcgtctccaggtactgtctgtcccagatcaagcctctgcacaacttcctgacccagctccagcccttcctgaagctcaagcagaagcaggccaacctcgtgctgaagatcatcgagcagctgccctccgccaaggaatccccggacaagttcctggaggtgtgcacctgggtggaccagatcgccgctctgaacgactccaagacccgcaagaccacttccgaaaccgtccgcgccgttctagacagtctctccgagaagaagaagtcgtccccctaaggtaccattcgagcagacatgataagatacattgatgagtttggacaaaccacaactagaatgcagtgaaaaaaatgctttatttgtgaaatttgtgatgctattgctttatttgtaaccattataagctgcaataaactagttcaatattggccattagccatattattcattggttatatagcataaatcaatattggctattggccattgcatacgttgtatctatatcataatatgtacatttatattggctcatgtccaatatgaccgccatgttggcattgattattgactagttattaatagtaatcaattacggggtcattagttcatagcccatatatggagttccgcgttacataacttacggtaaatggcccgcctggctgaccgcccaacgacccccgcccattgacgtcaataatgacgtatgttcccatagtaacgccaatagggactttccattgacgtcaatgggtggagtatttacggtaaactgcccacttggcagtacatcaagtgtatcatatgccaagtccgccccctattgacgtcaatgacggtaaatggcccgcctggcattatgcccagtacatgaccttacgggactttcctacttggcagtacatctacgtattagtcatcgctattaccatgatgatgcggttttggcagtacaccaatgggcgtggatagcggtttgactcacggggatttccaagtctccaccccattgacgtcaatgggagtttgttttggcaccaaaatcaacgggactttccaaaatgtcgtaataaccccgccccgttgacgcaaatgggcggtaggcgtgtacggtgggaggtctatataagcagagctcgtttagtgaaccgtcagatcactagaagcttaattgtgagcgctcacaattgtgagactgctgccgcagtcagtaattgtgagcgctcacaattgacctggagctgcaggagttggtaattgtgagcgctcacaattgcatgcgatatatatctaggccaccatggcccagtccaagcacggcctgaccaaggagatgaccatgaagtaccgcatggagggctgcgtggacggccacaagttcgtgatcaccggcgagggcatcggctaccccttcaagggcaagcaggtaagtatcaaggttacaagacaggtttaaggacatgcagccttctgtgatttgaggacatataagccggacttgtcgagacagagaagactcttgcgtttctgataggcacctattggtcttactgacatccactttgcctttctctccacaggccatcaacctgtgcgtggtggagggcggccccttgcccttcgccgaggacatcttgtccgccgccttcatgtacggcaaccgcgtgttcaccgagtacccccaggacatcgtcgactacttcaagaactcctgccccgccggctacacctgggaccgctccttcctgttcgaggacggcgccgtgtgcatctgcaacgccgacatcaccgtgagcgtggaggagaactgcatgtaccacgagtccaagttctacggcgtgaacttccccgccgacggccccgtgatgaagaagatgaccgacaactgggagccctcctgcgagaagatcatccccgtgcccaagcagggcatcttgaagggcgacgtgagcatgtacctgctgctgaaggacggtggccgcttgcgctgccagttcgacaccgtgtacaaggccaagtccgtgccccgcaagatgcccgactggcacttcatccagcacaagctgacccgcgaggaccgcagcgacgccaagaaccagaagtggcacctgaccgagcacgccatcgcctccggctccgccttgcccaagcttccgcggagccatggcttcccgccggcggtggcggcgcaggatgatggcacgctgcccatgtcttgtgcccaggagagcgggatggaccgtcaccctgcagcctgtgcttctgctaggatcaatgtgtagcggccgcaagcttggcgtaatcatggtcatagctgtttcctgtgtgaaattgttatccgctcacaattccacacaacatacgagccggaagcataaagtgtaaagcctggggtgcctaatgagtgagctaactcacattaattgcgttgcgctcactgcccgctttccagtcgggaaacctgtcgtgccagctgcattaatgaatcggccaacgcgcggggagaggcggtttgcgtattgggcgctcttccgcttcctcgctcactgactcgctgcgctcggtcgttcggctgcggcgagcggtatcagctcactcaaaggcggtaatacggttatccacagaatcaggggataacgcaggaaagaacatgtttattgcagcttataatggttacaaataaagcaatagcatcacaaatttcacaaataaagcatttttttcactgcattctagttgtggtttgtccaaactcatcaatgtatcttatcatgtctgctcgaagcggccgcggtacctcactgcccgctttccagtcgggaaacctgtcgtgccagctgcattaatgaatcggccaacgcgcggggagaggcggtttgcgtattgggcgccagggtggtttttcttttcaccagtgagacgggcaacagctgattgcccttcaccgcctggccctgagagagttgcagcaagcggtccacgctggtttgccccagcaggcgaaaatcctgtttgatggtggttaacggcgggatataacatgagctgtcttcggtatcgtcgtatcccactaccgagatatccgcaccaacgcgcagcccggactcggtaatggcgcgcattgcgcccagcgccatctgatcgttggcaaccagcatcgcagtgggaacgatgccctcattcagcatttgcatggtttgttgaaaaccggacatggcactccagtcgccttcccgttccgctatcggctgaatttgattgcgagtgagatatttatgccagccagccagacgcagacgcgccgagacagaacttaatgggcccgctaacagcgcgatttgctggtgacccaatgcgaccagatgctccacgcccagtcgcgtaccgtcttcatgggagaaaataatactgttgatgggtgtctggtcagagacatcaagaaataacgccggaacattagtgcaggcagcttccacagcaatggcatcctggtcatccagcggatagttaatgatcagcccactgacgcgttgcgcgagaagattgtgcaccgccgctttacaggcttcgacgccgcttcgttctaccatcgacaccaccacgctggcacccagttgatcggcgcgagatttaatcgccgcgacaatttgcgacggcgcgtgcagggccagactggaggtggcaacgccaatcagcaacgactgtttgcccgccagttgttgtgccacgcggttgggaatgtaattcagctccgccatcgccgcttccactttttcccgcgttttcgcagaaacgtggctggcctggttcaccacgcgggaaacggtctgataagagacaccggcatactctgcgacatcgtataacgttactggtttcaccatggtggctcgagctatagtgagtcgtattaagtactctagccttaagagctgtaattgaactgggagtggacacctgtggagagaaaggcaaagtggatgtcagtaagaccaataggtgcctatcagaaacgcaagagtcttctctgtctcgacaagcccagtttctattggtctccttaaacctgtcttgtaaccttgatacttacctgcccagtgcctcacgaccaacttctgcagcttaagttcgagactgttgtgtcagaagcactgactgcgttagcaatttaactgtgataaactaccgcaataaagcttctagtgatctgacggttcactaaacgagctctgcttatatagacctcccaccgtacacgcctaccgcccatttgcgtcaacggggcggggttattacgacattttggaaagtcccgttgattttggtgccaaaacaaactcccattgacgtcaatggggtggagacttggaaatccccgtgagtcaaaccgctatccacgcccattggtgtactgccaaaaccgcatcaccatggtaatagcgatgactaatacgtagatgtactgccaagtaggaaagtcccgtaaggtcatgtactgggcataatgccaggcgggccatttaccgtcattgacgtcaatagggggcggacttggcatatgatacacttgatgtactgccaagtgggcagtttaccgtaaatactccacccattgacgtcaatggaaagtccctattggcgttactatgggaacatacgtcattattgacgtcaatgggcgggggtcgttgggcggtcagccaggcgggccatttaccgtaagttatgtaacgcggaactccatatatgggctatgaactaatgaccccgtaattgattactattaataactagtcaataatcaatgccaacatggcggtcatattggacatgagccaatataaatgtacatattatgatatagatacaacgtatgcaatggccaatagccaatattgatttatgctatataaccaatgaataatatggctaatggccaatattgaacatgtgagcaaaaggccagcaaaaggccaggaaccgtaaaaaggccgcgttgctggcgtttttccataggctccgcccccctgacgagcatcacaaaaatcgacgctcaagtcagaggtggcgaaacccgacaggactataaagataccaggcgtttccccctggaagctccctcgtgcgctctcctgttccgaccctgccgcttaccggatacctgtccgcctttctcccttcgggaagcgtggcgctttctcatagctcacgctgtaggtatctcagttcggtgtaggtcgttcgctccaagctgggctgtgtgcacgaaccccccgttcagcccgaccgctgcgccttatccggtaactatcgtcttgagtccaacccggtaagacacgacttatcgccactggcagcagccactggtaacaggattagcagagcgaggtatgtaggcggtgctacagagttcttgaagtggtggcctaactacggctacactagaagaacagtatttggtatctgcgctctgctgaagccagttaccttcggaaaaagagttggtagctcttgatccggcaaacaaaccaccgctggtagcggtggtttttttgtttgcaagcagcagattacgcgcagaaaaaaaggatctcaagaagatcctttgatcttttctacggggtctgacgctcagtggaacgaaaactcacgttaagggattttggtcatgagattatcaaaaaggatcttcacctagatccttttaaattaaaaatgaagttttaaatcaatctaaagtatatatgagtaaacttggtctgacagttaccaatgcttaatcagtgaggcacctatctcagcgatctgtctatttcgttcatccatagttgcctgactccccgtcgtgtagataactacgatacgggagggcttaccatctggccccagtgctgcaatgataccgcgagacccacgctcaccggctccagatttatcagcaataaaccagccagccggaagggccgagcgcagaagtggtcctgcaactttatccgcctccatccagtctattaattgttgccgggaagctagagtaagtagttcgccagttaatagtttgcgcaacgttgttgccattgctacaggcatcgtggtgtcacgctcgtcgtttggtatggcttcattcagctccggttcccaacgatcaaggcgagttacatgatcccccatgttgtgcaaaaaagcggttagctccttcggtcctccgatcgttgtcagaagtaagttggccgcagtgttatcactcatggttatggcagcactgcataattctcttactgtcatgccatccgtaagatgcttttctgtgactggtgagtactcaaccaagtcattctgagaatagtgtatgcggcgaccgagttgctcttgcccggcgtcaatacgggataataccgcgccacatagcagaactttaaaagtgctcatcattggaaaacgttcttcggggcgaaaactctcaaggatcttaccgctgttgagatccagttcgatgtaacccactcgtgcacccaactgatcttcagcatcttttactttcaccagcgtttctgggtgagcaaaaacaggaaggcaaaatgccgcaaaaaagggaataagggcgacacggaaatgttgaatactcatactcttcctttttcaatattattgaagcatttatcagggttattgtctcatgagcggatacatatttgaatgtatttagaaaaataaacaaataggggttccgcgcacatttccccgaaaagtgccacctgacgtctaagaaaccattattatcatgacattaacctataaaaataggcgtatcacgaggccctttcgtc

SEQ ID NO: 5 - DNA, 6773 bp, Artificial Sequence
  Synthesized
tcgcgcgtttcggtgatgacggtgaaaacctctgacacatgcagctcccggagacggtcacagcttgtctgtaagcggatgccgggagcagacaagcccgtcagggcgcgtcagcgggtgttggcgggtgtcggggctggcttaactatgcggcatcagagcagattgtactgagagtgcaccatatgcggtgtgaaataccgcacagatgcgtaaggagaaaataccgcatcaggcgccattcgccattcaggctgcgcaactgttgggaagggcgatcggtgcgggcctcttcgctattacgccagctggcgaaagggggatgtgctgcaaggcgattaagttgggtaacgccagggttttcccagtcacgacgttgtaaaacgacggccagtgaattcagatcttcaatattggccattagccatattattcattggttatatagcataaatcaatattggctattggccattgcatacgttgtatctatatcataatatgtacatttatattggctcatgtccaatatgaccgccatgttggcattgattattgactagttattaatagtaatcaattacggggtcattagttcatagcccatatatggagttccgcgttacataacttacggtaaatggcccgcctggctgaccgcccaacgacccccgcccattgacgtcaataatgacgtatgttcccatagtaacgccaatagggactttccattgacgtcaatgggtggagtatttacggtaaactgcccacttggcagtacatcaagtgtatcatatgccaagtccgccccctattgacgtcaatgacggtaaatggcccgcctggcattatgcccagtacatgaccttacgggactttcctacttggcagtacatctacgtattagtcatcgctattaccatgatgatgcggttttggcagtacaccaatgggcgtggatagcggtttgactcacggggatttccaagtctccaccccattgacgtcaatgggagtttgttttggcaccaaaatcaacgggactttccaaaatgtcgtaataaccccgccccgttgacgcaaatgggcggtaggcgtgtacggtgggaggtctatataagcagagctcgtttagtgaaccgtcagatcactagaagcttaattgtgagcgctcacaattgtgagactgctgccgcagtcagtaattgtgagcgctcacaattgacctggagctgcaggagttggtaattgtgagcgctcacaattctcgagatatatatctaggccaccatggcaccgaagaagaagcgcaaggtgcatatgaatacaaaatataataaggtaagtatcaaggttacaagacaggtttaaggcgccaatagaagcttggcttgtcgagacagagaagactcttgcgtttctgataggcacctattggtcttactgacatccactttgcctttctctccacaggagttcttactctacttagcagggtttgtagacggtgacggttccatctttgcctgtatccatcctagtcaagcgtataagttcaagcaccggctgactctccatttcacggtcactcagaagacacagcgccgttggttcctcgacaagctggtggacgagatcggtgtgggttacgtgcaggacgtgggcagcgtctcccagtaccggctgtcccagatcaagcctttgcataattttttaacacaactacaaccttttctaaaactaaaacaaaaacaagcaaatttagttttaaaaattattgaacaacttccgtcagcaaaagaatccccggacaaattcttagaagtttgtacatgggtggatcaaattgcagctctgaatgattcgaagacgcgtaaaacaacttctgaaaccgttcgtgctgtgctagacagtttaccaggatccgtgggaggtctatcgccatctcaggcatccagcgccgcatcctcggcttcctcaagcccgggttcagggatctccgaagcactcagagctggagcaggttccggcactggatacaacaaggaattcctgctctacctggcgggcttcgtcgacggggacggctccatctctgccactatcgctccggctcagtatggtaagttcaagcactatctggggctccggttctatgtcagtcagaagacacagcgccgttggttcctcgacaagctggtggacgagatcggtgtgggttacgtgagtgaccagggcagcgtctccaggtactgtctgtcccagatcaagcctctgcacaacttcctgacccagctccagcccttcctgaagctcaagcagaagcaggccaacctcgtgctgaagatcatcgagcagctgccctccgccaaggaatccccggacaagttcctggaggtgtgcacctgggtggaccagatcgccgctctgaacgactccaagacccgcaagaccacttccgaaaccgtccgcgccgttctagacagtctctccgagaagaagaagtcgtccccctaaggtaccattcgagcagacatgataagatacattgatgagtttggacaaaccacaactagaatgcagtgaaaaaaatgctttatttgtgaaatttgtgatgctattgctttatttgtaaccattataagctgcaataaactagttcaatattggccattagccatattattcattggttatatagcataaatcaatattggctattggccattgcatacgttgtatctatatcataatatgtacatttatattggctcatgtccaatatgaccgccatgttggcattgattattgactagttattaatagtaatcaattacggggtcattagttcatagcccatatatggagttccgcgttacataacttacggtaaatggcccgcctggctgaccgcccaacgacccccgcccattgacgtcaataatgacgtatgttcccatagtaacgccaatagggactttccattgacgtcaatgggtggagtatttacggtaaactgcccacttggcagtacatcaagtgtatcatatgccaagtccgccccctattgacgtcaatgacggtaaatggcccgcctggcattatgcccagtacatgaccttacgggactttcctacttggcagtacatctacgtattagtcatcgctattaccatgatgatgcggttttggcagtacaccaatgggcgtggatagcggtttgactcacggggatttccaagtctccaccccattgacgtcaatgggagtttgttttggcaccaaaatcaacgggactttccaaaatgtcgtaataaccccgccccgttgacgcaaatgggcggtaggcgtgtacggtgggaggtctatataagcagagctcgtttagtgaaccgtcagatcactagaagcttaattgtgagcgctcacaattgtgagactgctgccgcagtcagtaattgtgagcgctcacaattgacctggagctgcaggagttggtaattgtgagcgctcacaattgcatgcgatatatatctaggccaccatggcccagtccaagcacggcctgaccaaggagatgaccatgaagtaccgcatggagggctgcgtggacggccacaagttcgtgatcaccggcgagggcatcggctaccccttcaagggcaagcaggtaagtatcaaggttacaagacaggtttaaggacatgcagccttctgtgatttgaggacatataagccggacttgtcgagacagagaagactcttgcgtttctgataggcacctattggtcttactgacatccactttgcctttctctccacaggccatcaacctgtgcgtggtggagggcggccccttgcccttcgccgaggacatcttgtccgccgccttcatgtacggcaaccgcgtgttcaccgagtacccccaggacatcgtcgactacttcaagaactcctgccccgccggctacacctgggaccgctccttcctgttcgaggacggcgccgtgtgcatctgcaacgccgacatcaccgtgagcgtggaggagaactgcatgtaccacgagtccaagttctacggcgtgaacttccccgccgacggccccgtgatgaagaagatgaccgacaactgggagccctcctgcgagaagatcatccccgtgcccaagcagggcatcttgaagggcgacgtgagcatgtacctgctgctgaaggacggtggccgcttgcgctgccagttcgacaccgtgtacaaggccaagtccgtgccccgcaagatgcccgactggcacttcatccagcacaagctgacccgcgaggaccgcagcgacgccaagaaccagaagtggcacctgaccgagcacgccatcgcctccggctccgccttgcccaagcttccgcggagccatggcttcccgccggcggtggcggcgcaggatgatggcacgctgcccatgtcttgtgcccaggagagcgggatggaccgtcaccctgcagcctgtgcttctgctaggatcaatgtgtagcggccgcaagcttggcgtaatcatggtcatagctgtttcctgtgtgaaattgttatccgctcacaattccacacaacatacgagccggaagcataaagtgtaaagcctggggtgcctaatgagtgagctaactcacattaattgcgttgcgctcactgcccgctttccagtcgggaaacctgtcgtgccagctgcattaatgaatcggccaacgcgcggggagaggcggtttgcgtattgggcgctcttccgcttcctcgctcactgactcgctgcgctcggtcgttcggctgcggcgagcggtatcagctcactcaaaggcggtaatacggttatccacagaatcaggggataacgcaggaaagaacatgtgagcaaaaggccagcaaaaggccaggaaccgtaaaaaggccgcgttgctggcgtttttccataggctccgcccccctgacgagcatcacaaaaatcgacgctcaagtcagaggtggcgaaacccgacaggactataaagataccaggcgtttccccctggaagctccctcgtgcgctctcctgttccgaccctgccgcttaccggatacctgtccgcctttctcccttcgggaagcgtggcgctttctcatagctcacgctgtaggtatctcagttcggtgtaggtcgttcgctccaagctgggctgtgtgcacgaaccccccgttcagcccgaccgctgcgccttatccggtaactatcgtcttgagtccaacccggtaagacacgacttatcgccactggcagcagccactggtaacaggattagcagagcgaggtatgtaggcggtgctacagagttcttgaagtggtggcctaactacggctacactagaagaacagtatttggtatctgcgctctgctgaagccagttaccttcggaaaaagagttggtagctcttgatccggcaaacaaaccaccgctggtagcggtggtttttttgtttgcaagcagcagattacgcgcagaaaaaaaggatctcaagaagatcctttgatcttttctacggggtctgacgctcagtggaacgaaaactcacgttaagggattttggtcatgagattatcaaaaaggatcttcacctagatccttttaaattaaaaatgaagttttaaatcaatctaaagtatatatgagtaaacttggtctgacagttaccaatgcttaatcagtgaggcacctatctcagcgatctgtctatttcgttcatccatagttgcctgactccccgtcgtgtagataactacgatacgggagggcttaccatctggccccagtgctgcaatgataccgcgagacccacgctcaccggctccagatttatcagcaataaaccagccagccggaagggccgagcgcagaagtggtcctgcaactttatccgcctccatccagtctattaattgttgccgggaagctagagtaagtagttcgccagttaatagtttgcgcaacgttgttgccattgctacaggcatcgtggtgtcacgctcgtcgtttggtatggcttcattcagctccggttcccaacgatcaaggcgagttacatgatcccccatgttgtgcaaaaaagcggttagctccttcggtcctccgatcgttgtcagaagtaagttggccgcagtgttatcactcatggttatggcagcactgcataattctcttactgtcatgccatccgtaagatgcttttctgtgactggtgagtactcaaccaagtcattctgagaatagtgtatgcggcgaccgagttgctcttgcccggcgtcaatacgggataataccgcgccacatagcagaactttaaaagtgctcatcattggaaaacgttcttcggggcgaaaactctcaaggatcttaccgctgttgagatccagttcgatgtaacccactcgtgcacccaactgatcttcagcatcttttactttcaccagcgtttctgggtgagcaaaaacaggaaggcaaaatgccgcaaaaaagggaataagggcgacacggaaatgttgaatactcatactcttcctttttcaatattattgaagcatttatcagggttattgtctcatgagcggatacatatttgaatgtatttagaaaaataaacaaataggggttccgcgcacatttccccgaaaagtgccacctgacgtctaagaaaccattattatcatgacattaacctataaaaataggcgtatcacgaggccctttcgtc

SEQ ID NO: 6 - DNA, 5741 bp, Artificial Sequence
  Synthesized
cagcagctggcgtaatagcgaagaggcccgcaccgatcgcccttcccaacagttgcgcagcctgaatggcgaatggaattccagacgattgagcgtcaaaatgtaggtatttccatgagcgtttttcctgttgcaatggctggcggtaatattgttctggatattaccagcaaggccgatagtttgagttcttctactcaggcaagtgatgttattactaatcaaagaagtattgcgacaacggttaatttgcgtgatggacagactcttttactcggtggcctcactgattataaaaacacttctcaggattctggcgtaccgttcctgtctaaaatccctttaatcggcctcctgtttagctcccgctctgattctaacgaggaaagcacgttatacgtgctcgtcaaagcaaccatagtacgcgccctgtagcggcgcattaagcgcggcgggtgtggtggttacgcgcagcgtgaccgctacacttgccagcgccctagcgcccgctcctttcgctttcttcccttcctttctcgccacgttcgccggctttccccgtcaagctctaaatcgggggctccctttagggttccgatttagtgctttacggcacctcgaccccaaaaaacttgattagggtgatggttcacgtagtgggccatcgccctgatagacggtttttcgccctttgacgttggagtccacgttctttaatagtggactcttgttccaaactggaacaacactcaaccctatctcggtctattcttttgatttataagggattttgccgatttcggcctattggttaaaaaatgagctgatttaacaaaaatttaacgcgaattttaacaaaatattaacgtttacaatttaaatatttgcttatacaatcttcctgtttttggggcttttctgattatcaaccggggtacatatgattgacatgctagttttacgattaccgttcatcgccctgcgcgctcgctcgctcactgaggccgcccgggcaaagcccgggcgtcgggcgacctttggtcgcccggcctcagtgagcgagcgagcgcgcagagagggagtggaattcacgcgtgggccccagaagcctggtggttgtttgtccttctcaggggaaaagtgaggcggccccttggaggaaggggccgggcagaatgatctaatcggattccaagcagctcaggggattgtctttttctagcaccttcttgccactcctaagcgtcctccgtgaccccggctgggatttagcctggtgctgtgtcagccccgggctcccaggggcttcccagtggtccccaggaaccctcgacagggccagggcgtctctctcgtccagcaagggcagggacgggccacaggccaagggcaagcttggctagccaccatggcaccgaagaagaagcgcaaggtgcatatgaatacaaaatataataaggtaagtatcaaggttacaagacaggtttaaggcgccaatagaaacgggtgtggtacgcagccactggcttgtcgagacagagaagactcttgcgtttctgataggcacctattggtcttactgacatccactttgcctttctctccacaggagttcttactctacttagcagggtttgtagacggtgacggttccatctatgcccgtatctttaagggtcaacattggaagttcaagcactatattcgtttgaccttctgtgtgcggcagaagacacagcgccgttggttcctcgacaagctggtggacgagatcggtgtgggttacgtgactgactctggcagcgtttccgcttactatctgtccgagatcaagcctttgcataattttttaacacaactacaaccttttctaaaactaaaacaaaaacaagcaaatttagttttaaaaattattgaacaacttccgtcagcaaaagaatccccggacaaattcttagaagtttgtacatgggtggatcaaattgcagctctgaatgattcgaagacgcgtaaaacaacttctgaaaccgttcgtgctgtgctagacagtttaccaggatccgtgggaggtctatcgccatctcaggcatccagcgccgcatcctcggcttcctcaagcccgggttcagggatctccgaagcactcagagctggagcaggttccggcactggatacaacaaggaattcctgctctacctggcgggcttcgtcgacggggacggctccatctgggcctcgatcattcctgagcaaggttataagttcaagcacaggctgcgtctctctttcactgtcgctcagaagacacagcgccgttggttcctcgacaagctggtggacgagatcggtgtgggttacgtggttgaccagggcagcgtctccgagtacaggctgtccgagatcaagcctctgcacaacttcctgacccagctccagcccttcctgaagctcaagcagaagcaggccaacctcgtgctgaagatcatcgagcagctgccctccgccaaggaatccccggacaagttcctggaggtgtgcacctgggtggaccagatcgccgctctgaacgactccaagacccgcaagaccacttccgaaaccgtccgcgccgttctagacagtctctccgagaagaagaagtcgtccccctaagcggccgcgactctagatcataatcagccataccacatttgtagaggttttacttgctttaaaaaacctcccacacctccccctgaacctgaaacataaaatgaatgcaattgttgttgttaacttgtttattgcagcttataatggttacaaataaagcaatagcatcacaaatttcacaaataaagcatttttttcactgcattctagttgtggtttgtccaaactcatcaatgtatcttaaggcgggaattgatctaggaacccctagtgatggagttggccactccctctctgcgcgctcgctcgctcactgaggccgcccgggcaaagcccgggcgtcgggcgacctttggtcgcccggcctcagtgagcgagcgagcgcgcagagagggagtggccaaccccccccccccccccccggcgattctcttgtttgctccagactctcaggcaatgacctgatagcctttgtagagacctctcaaaaatagctaccctctccggcatgaatttatcagctagaacggttgaatatcatattgatggtgatttgactgtctccggcctttctcacccgtttgaatctttacctacacattactcaggcattgcatttaaaatatatgagggttctaaaaatttttatccttgcgttgaaataaaggcttctcccgcaaaagtattacagggtcataatgtttttggtacaaccgatttagctttatgctctgaggctttattgcttaattttgctaattctttgccttgcctgtatgatttattggatgttggaattcctgatgcggtattttctccttacgcatctgtgcggtatttcacaccgcatatggtgcactctcagtacaatctgctctgatgccgcatagttaagccagccccgacacccgccaacacccgctgacgcgccctgacgggcttgtctgctcccggcatccgcttacagacaagctgtgaccgtctccgggagctgcatgtgtcagaggttttcaccgtcatcaccgaaacgcgcgagacgaaagggcctcgtgatacgcctatttttataggttaatgtcatgataataatggtttcttagacgtcaggtggcacttttcggggaaatgtgcgcggaacccctatttgtttatttttctaaatacattcaaatatgtatccgctcatgagacaataaccctgataaatgcttcaataatattgaaaaaggaagagtatgagtattcaacatttccgtgtcgcccttattcccttttttgcggcattttgccttcctgtttttgctcacccagaaacgctggtgaaagtaaaagatgctgaagatcagttgggtgcacgagtgggttacatcgaactggatctcaacagcggtaagatccttgagagttttcgccccgaagaacgttttccaatgatgagcacttttaaagttctgctatgtggcgcggtattatcccgtattgacgccgggcaagagcaactcggtcgccgcatacactattctcagaatgacttggttgagtactcaccagtcacagaaaagcatcttacggatggcatgacagtaagagaattatgcagtgctgccataaccatgagtgataacactgcggccaacttacttctgacaacgatcggaggaccgaaggagctaaccgcttttttgcacaacatgggggatcatgtaactcgccttgatcgttgggaaccggagctgaatgaagccataccaaacgacgagcgtgacaccacgatgcctgtagcaatggcaacaacgttgcgcaaactattaactggcgaactacttactctagcttcccggcaacaattaatagactggatggaggcggataaagttgcaggaccacttctgcgctcggcccttccggctggctggtttattgctgataaatctggagccggtgagcgtgggtctcgcggtatcattgcagcactggggccagatggtaagccctcccgtatcgtagttatctacacgacggggagtcaggcaactatggatgaacgaaatagacagatcgctgagataggtgcctcactgattaagcattggtaactgtcagaccaagtttactcatatatactttagattgatttaaaacttcatttttaatttaaaaggatctaggtgaagatcctttttgataatctcatgaccaaaatcccttaacgtgagttttcgttccactgagcgtcagaccccgtagaaaagatcaaaggatcttcttgagatcctttttttctgcgcgtaatctgctgcttgcaaacaaaaaaaccaccgctaccagcggtggtttgtttgccggatcaagagctaccaactctttttccgaaggtaactggcttcagcagagcgcagataccaaatactgtccttctagtgtagccgtagttaggccaccacttcaagaactctgtagcaccgcctacatacctcgctctgctaatcctgttaccagtggctgctgccagtggcgataagtcgtgtcttaccgggttggactcaagacgatagttaccggataaggcgcagcggtcgggctgaacggggggttcgtgcacacagcccagcttggagcgaacgacctacaccgaactgagatacctacagcgtgagctatgagaaagcgccacgcttcccgaagggagaaaggcggacaggtatccggtaagcggcagggtcggaacaggagagcgcacgagggagcttccagggggaaacgcctggtatctttatagtcctgtcgggtttcgccacctctgacttgagcgtcgatttttgtgatgctcgtcaggggggcggagcctatggaaaaacgccagcaacgcggcctttttacggttcctggccttttgctggccttttgctcacatgttctttcctgcgttatcccctgattctgtggataaccgtattaccgcctttgagtgagctgataccgctcgccgcagccgaacgaccgagcgcagcgagtcagtgagcgaggaagcggaagagcgcccaatacgcaaaccgcctctccccgcgcgttggccgattcattaatg

SEQ ID NO: 7 - DNA, 6335 bp, Artificial Sequence
  Synthesized
cagcagctggcgtaatagcgaagaggcccgcaccgatcgcccttcccaacagttgcgcagcctgaatggcgaatggaattccagacgattgagcgtcaaaatgtaggtatttccatgagcgtttttcctgttgcaatggctggcggtaatattgttctggatattaccagcaaggccgatagtttgagttcttctactcaggcaagtgatgttattactaatcaaagaagtattgcgacaacggttaatttgcgtgatggacagactcttttactcggtggcctcactgattataaaaacacttctcaggattctggcgtaccgttcctgtctaaaatccctttaatcggcctcctgtttagctcccgctctgattctaacgaggaaagcacgttatacgtgctcgtcaaagcaaccatagtacgcgccctgtagcggcgcattaagcgcggcgggtgtggtggttacgcgcagcgtgaccgctacacttgccagcgccctagcgcccgctcctttcgctttcttcccttcctttctcgccacgttcgccggctttccccgtcaagctctaaatcgggggctccctttagggttccgatttagtgctttacggcacctcgaccccaaaaaacttgattagggtgatggttcacgtagtgggccatcgccctgatagacggtttttcgccctttgacgttggagtccacgttctttaatagtggactcttgttccaaactggaacaacactcaaccctatctcggtctattcttttgatttataagggattttgccgatttcggcctattggttaaaaaatgagctgatttaacaaaaatttaacgcgaattttaacaaaatattaacgtttacaatttaaatatttgcttatacaatcttcctgtttttggggcttttctgattatcaaccggggtacatatgattgacatgctagttttacgattaccgttcatcgccctgcgcgctcgctcgctcactgaggccgcccgggcaaagcccgggcgtcgggcgacctttggtcgcccggcctcagtgagcgagcgagcgcgcagagagggagtggaattcacgcgtggatcttaatagtaatcaattacggggtcattagttcatagcccatatatggagttccgcgttacataacttacggtaaatggcccgcctggctgaccgcccaacgacccccgcccattgacgtcaataatgacgtatgttcccatagtaacgccaatagggactttccattgacgtcaatgggtggagtatttacggtaaactgcccacttggcagtacatcaagtgtatcatatgccaagtccgccccctattgacgtcaatgacggtaaatggcccgcctggcattatgcccagtacatgaccttacgggactttcctacttggcagtacatctacgtattagtcatcgctattaccatggtgatgcggttttggcagtacaccaatgggcgtggatagcggtttgactcacggggatttccaagtctccaccccattgacgtcaatgggagtttgttttggcaccaaaatcaacgggactttccaaaatgtcgtaataaccccgccccgttgacgcaaatgggcggtaggcgtgtacggtgggaggtctatataagcagagctcgtttagtgaaccgtcagatcactagaagctttattgcggtagtttatcacagttaaattgctaacgcagtcagtgcttctgacacaacagtctcgaacttaagctgcagaagttggtcgtgaggcactgggcaggtgtccactcccagttcaattacagctcttaaggctagagtacttaatacgactcactataggctagccaccatggcaccgaagaagaagcgcaaggtgcatatgaatacaaaatataataaagagttcttactctacttagcagggtaagcgcccctaaaatccctttgggcacaatgtgtcctgaggggagaggcagcgacctgtagatgggacacgggtgtggtacgcagccactgggggcactaaccctcaggtttggggcttctgaatgtgagtatcgccatgtaagcccagtatttggccaatctcagaaagctcctggtccctggagggatggagagagaaaaacaaacagctcctggagcagggagagtgctggcctcttgctctccggctccctctgttgccctctggtttctccccaggtttgtagacggtgacggttccatctatgcccgtatctttaagggtcaacattggaagttcaagcactatattcgtttgaccttctgtgtgcggcagaagacacagcgccgttggttcctcgacaagctggtggacgagatcggtgtgggttacgtgactgactctggcagcgtttccgcttactatctgtccgagatcaagcctttgcataattttttaacacaactacaaccttttctaaaactaaaacaaaaacaagcaaatttagttttaaaaattattgaacaacttccgtcagcaaaagaatccccggacaaattcttagaagtttgtacatgggtggatcaaattgcagctctgaatgattcgaagacgcgtaaaacaacttctgaaaccgttcgtgctgtgctagacagtttaccaggatccgtgggaggtctatcgccatctcaggcatccagcgccgcatcctcggcttcctcaagcccgggttcagggatctccgaagcactcagagctggagcaggttccggcactggatacaacaaggaattcctgctctacctggcgggcttcgtcgacggggacggctccatctgggcctcgatcattcctgagcaaggttataagttcaagcacaggctgcgtctctctttcactgtcgctcagaagacacagcgccgttggttcctcgacaagctggtggacgagatcggtgtgggttacgtggttgaccagggcagcgtctccgagtacaggctgtccgagatcaagcctctgcacaacttcctgacccagctccagcccttcctgaagctcaagcagaagcaggccaacctcgtgctgaagatcatcgagcagctgccctccgccaaggaatccccggacaagttcctggaggtgtgcacctgggtggaccagatcgccgctctgaacgactccaagacccgcaagaccacttccgaaaccgtccgcgccgttctagacagtctctccgagaagaagaagtcgtccccctaagcggccgcgactctagatcataatcagccataccacatttgtagaggttttacttgctttaaaaaacctcccacacctccccctgaacctgaaacataaaatgaatgcaattgttgttgttaacttgtttattgcagcttataatggttacaaataaagcaatagcatcacaaatttcacaaataaagcatttttttcactgcattctagttgtggtttgtccaaactcatcaatgtatcttaaggcgggaattgatctaggaacccctagtgatggagttggccactccctctctgcgcgctcgctcgctcactgaggccgcccgggcaaagcccgggcgtcgggcgacctttggtcgcccggcctcagtgagcgagcgagcgcgcagagagggagtggccaaccccccccccccccccccggcgattctcttgtttgctccagactctcaggcaatgacctgatagcctttgtagagacctctcaaaaatagctaccctctccggcatgaatttatcagctagaacggttgaatatcatattgatggtgatttgactgtctccggcctttctcacccgtttgaatctttacctacacattactcaggcattgcatttaaaatatatgagggttctaaaaatttttatccttgcgttgaaataaaggcttctcccgcaaaagtattacagggtcataatgtttttggtacaaccgatttagctttatgctctgaggctttattgcttaattttgctaattctttgccttgcctgtatgatttattggatgttggaattcctgatgcggtattttctccttacgcatctgtgcggtatttcacaccgcatatggtgcactctcagtacaatctgctctgatgccgcatagttaagccagccccgacacccgccaacacccgctgacgcgccctgacgggcttgtctgctcccggcatccgcttacagacaagctgtgaccgtctccgggagctgcatgtgtcagaggttttcaccgtcatcaccgaaacgcgcgagacgaaagggcctcgtgatacgcctatttttataggttaatgtcatgataataatggtttcttagacgtcaggtggcacttttcggggaaatgtgcgcggaacccctatttgtttatttttctaaatacattcaaatatgtatccgctcatgagacaataaccctgataaatgcttcaataatattgaaaaaggaagagtatgagtattcaacatttccgtgtcgcccttattcccttttttgcggcattttgccttcctgtttttgctcacccagaaacgctggtgaaagtaaaagatgctgaagatcagttgggtgcacgagtgggttacatcgaactggatctcaacagcggtaagatccttgagagttttcgccccgaagaacgttttccaatgatgagcacttttaaagttctgctatgtggcgcggtattatcccgtattgacgccgggcaagagcaactcggtcgccgcatacactattctcagaatgacttggttgagtactcaccagtcacagaaaagcatcttacggatggcatgacagtaagagaattatgcagtgctgccataaccatgagtgataacactgcggccaacttacttctgacaacgatcggaggaccgaaggagctaaccgcttttttgcacaacatgggggatcatgtaactcgccttgatcgttgggaaccggagctgaatgaagccataccaaacgacgagcgtgacaccacgatgcctgtagcaatggcaacaacgttgcgcaaactattaactggcgaactacttactctagcttcccggcaacaattaatagactggatggaggcggataaagttgcaggaccacttctgcgctcggcccttccggctggctggtttattgctgataaatctggagccggtgagcgtgggtctcgcggtatcattgcagcactggggccagatggtaagccctcccgtatcgtagttatctacacgacggggagtcaggcaactatggatgaacgaaatagacagatcgctgagataggtgcctcactgattaagcattggtaactgtcagaccaagtttactcatatatactttagattgatttaaaacttcatttttaatttaaaaggatctaggtgaagatcctttttgataatctcatgaccaaaatcccttaacgtgagttttcgttccactgagcgtcagaccccgtagaaaagatcaaaggatcttcttgagatcctttttttctgcgcgtaatctgctgcttgcaaacaaaaaaaccaccgctaccagcggtggtttgtttgccggatcaagagctaccaactctttttccgaaggtaactggcttcagcagagcgcagataccaaatactgtccttctagtgtagccgtagttaggccaccacttcaagaactctgtagcaccgcctacatacctcgctctgctaatcctgttaccagtggctgctgccagtggcgataagtcgtgtcttaccgggttggactcaagacgatagttaccggataaggcgcagcggtcgggctgaacggggggttcgtgcacacagcccagcttggagcgaacgacctacaccgaactgagatacctacagcgtgagctatgagaaagcgccacgcttcccgaagggagaaaggcggacaggtatccggtaagcggcagggtcggaacaggagagcgcacgagggagcttccagggggaaacgcctggtatctttatagtcctgtcgggtttcgccacctctgacttgagcgtcgatttttgtgatgctcgtcaggggggcggagcctatggaaaaacgccagcaacgcggcctttttacggttcctggccttttgctggccttttgctcacatgttctttcctgcgttatcccctgattctgtggataaccgtattaccgcctttgagtgagctgataccgctcgccgcagccgaacgaccgagcgcagcgagtcagtgagcgaggaagcggaagagcgcccaatacgcaaaccgcctctccccgcgcgttggccgattcattaatg

SEQ ID NO: 8 - DNA, 6421 bp, Artificial Sequence
  Synthesized
cagcagctggcgtaatagcgaagaggcccgcaccgatcgcccttcccaacagttgcgcagcctgaatggcgaatggaattccagacgattgagcgtcaaaatgtaggtatttccatgagcgtttttcctgttgcaatggctggcggtaatattgttctggatattaccagcaaggccgatagtttgagttcttctactcaggcaagtgatgttattactaatcaaagaagtattgcgacaacggttaatttgcgtgatggacagactcttttactcggtggcctcactgattataaaaacacttctcaggattctggcgtaccgttcctgtctaaaatccctttaatcggcctcctgtttagctcccgctctgattctaacgaggaaagcacgttatacgtgctcgtcaaagcaaccatagtacgcgccctgtagcggcgcattaagcgcggcgggtgtggtggttacgcgcagcgtgaccgctacacttgccagcgccctagcgcccgctcctttcgctttcttcccttcctttctcgccacgttcgccggctttccccgtcaagctctaaatcgggggctccctttagggttccgatttagtgctttacggcacctcgaccccaaaaaacttgattagggtgatggttcacgtagtgggccatcgccctgatagacggtttttcgccctttgacgttggagtccacgttctttaatagtggactcttgttccaaactggaacaacactcaaccctatctcggtctattcttttgatttataagggattttgccgatttcggcctattggttaaaaaatgagctgatttaacaaaaatttaacgcgaattttaacaaaatattaacgtttacaatttaaatatttgcttatacaatcttcctgtttttggggcttttctgattatcaaccggggtacatatgattgacatgctagttttacgattaccgttcatcgccctgcgcgctcgctcgctcactgaggccgcccgggcaaagcccgggcgtcgggcgacctttggtcgcccggcctcagtgagcgagcgagcgcgcagagagggagtggaattcacgcgtggatcttaatagtaatcaattacggggtcattagttcatagcccatatatggagttccgcgttacataacttacggtaaatggcccgcctggctgaccgcccaacgacccccgcccattgacgtcaataatgacgtatgttcccatagtaacgccaatagggactttccattgacgtcaatgggtggagtatttacggtaaactgcccacttggcagtacatcaagtgtatcatatgccaagtccgccccctattgacgtcaatgacggtaaatggcccgcctggcattatgcccagtacatgaccttacgggactttcctacttggcagtacatctacgtattagtcatcgctattaccatggtgatgcggttttggcagtacaccaatgggcgtggatagcggtttgactcacggggatttccaagtctccaccccattgacgtcaatgggagtttgttttggcaccaaaatcaacgggactttccaaaatgtcgtaataaccccgccccgttgacgcaaatgggcggtaggcgtgtacggtgggaggtctatataagcagagctcgtttagtgaaccgtcagatcactagaagctttattgcggtagtttatcacagttaaattgctaacgcagtcagtgcttctgacacaacagtctcgaacttaagctgcagaagttggtcgtgaggcactgggcaggtgtccactcccagttcaattacagctcttaaggctagagtacttaatacgactcactataggctagccaccatggcaccgaagaagaagcgcaaggtgcatatgaatacaaaatataataaagagttcttactctacttagcagggtatttgcttcttccttaaatcctggtgttgatgcaatgtactgcaaacaatggcctgagtgtgcaaagaaaatgtctgctaactgcatatgcttgctgtgcttactgaggatgaagcatgaaaatagaaaattatacaggaaagatccacttgtgtgggttgattgctactgcttcgattgctttagaatgtggtttggacgggtgtggtacgcagccactacttgatctttgtgaaggaaccttacttctgtggtgtgacataattggacaaactacctacagagatttaaagctctaaggtaaatataaaatttttaagtgtataatgtgttaaactactgattctaattgtttgtgtattttaggtttgtagacggtgacggttccatctatgcccgtatctttaagggtcaacattggaagttcaagcactatattcgtttgaccttctgtgtgcggcagaagacacagcgccgttggttcctcgacaagctggtggacgagatcggtgtgggttacgtgactgactctggcagcgtttccgcttactatctgtccgagatcaagcctttgcataattttttaacacaactacaaccttttctaaaactaaaacaaaaacaagcaaatttagttttaaaaattattgaacaacttccgtcagcaaaagaatccccggacaaattcttagaagtttgtacatgggtggatcaaattgcagctctgaatgattcgaagacgcgtaaaacaacttctgaaaccgttcgtgctgtgctagacagtttaccaggatccgtgggaggtctatcgccatctcaggcatccagcgccgcatcctcggcttcctcaagcccgggttcagggatctccgaagcactcagagctggagcaggttccggcactggatacaacaaggaattcctgctctacctggcgggcttcgtcgacggggacggctccatctgggcctcgatcattcctgagcaaggttataagttcaagcacaggctgcgtctctctttcactgtcgctcagaagacacagcgccgttggttcctcgacaagctggtggacgagatcggtgtgggttacgtggttgaccagggcagcgtctccgagtacaggctgtccgagatcaagcctctgcacaacttcctgacccagctccagcccttcctgaagctcaagcagaagcaggccaacctcgtgctgaagatcatcgagcagctgccctccgccaaggaatccccggacaagttcctggaggtgtgcacctgggtggaccagatcgccgctctgaacgactccaagacccgcaagaccacttccgaaaccgtccgcgccgttctagacagtctctccgagaagaagaagtcgtccccctaagcggccgcgactctagatcataatcagccataccacatttgtagaggttttacttgctttaaaaaacctcccacacctccccctgaacctgaaacataaaatgaatgcaattgttgttgttaacttgtttattgcagcttataatggttacaaataaagcaatagcatcacaaatttcacaaataaagcatttttttcactgcattctagttgtggtttgtccaaactcatcaatgtatcttaaggcgggaattgatctaggaacccctagtgatggagttggccactccctctctgcgcgctcgctcgctcactgaggccgcccgggcaaagcccgggcgtcgggcgacctttggtcgcccggcctcagtgagcgagcgagcgcgcagagagggagtggccaaccccccccccccccccccggcgattctcttgtttgctccagactctcaggcaatgacctgatagcctttgtagagacctctcaaaaatagctaccctctccggcatgaatttatcagctagaacggttgaatatcatattgatggtgatttgactgtctccggcctttctcacccgtttgaatctttacctacacattactcaggcattgcatttaaaatatatgagggttctaaaaatttttatccttgcgttgaaataaaggcttctcccgcaaaagtattacagggtcataatgtttttggtacaaccgatttagctttatgctctgaggctttattgcttaattttgctaattctttgccttgcctgtatgatttattggatgttggaattcctgatgcggtattttctccttacgcatctgtgcggtatttcacaccgcatatggtgcactctcagtacaatctgctctgatgccgcatagttaagccagccccgacacccgccaacacccgctgacgcgccctgacgggcttgtctgctcccggcatccgcttacagacaagctgtgaccgtctccgggagctgcatgtgtcagaggttttcaccgtcatcaccgaaacgcgcgagacgaaagggcctcgtgatacgcctatttttataggttaatgtcatgataataatggtttcttagacgtcaggtggcacttttcggggaaatgtgcgcggaacccctatttgtttatttttctaaatacattcaaatatgtatccgctcatgagacaataaccctgataaatgcttcaataatattgaaaaaggaagagtatgagtattcaacatttccgtgtcgcccttattcccttttttgcggcattttgccttcctgtttttgctcacccagaaacgctggtgaaagtaaaagatgctgaagatcagttgggtgcacgagtgggttacatcgaactggatctcaacagcggtaagatccttgagagttttcgccccgaagaacgttttccaatgatgagcacttttaaagttctgctatgtggcgcggtattatcccgtattgacgccgggcaagagcaactcggtcgccgcatacactattctcagaatgacttggttgagtactcaccagtcacagaaaagcatcttacggatggcatgacagtaagagaattatgcagtgctgccataaccatgagtgataacactgcggccaacttacttctgacaacgatcggaggaccgaaggagctaaccgcttttttgcacaacatgggggatcatgtaactcgccttgatcgttgggaaccggagctgaatgaagccataccaaacgacgagcgtgacaccacgatgcctgtagcaatggcaacaacgttgcgcaaactattaactggcgaactacttactctagcttcccggcaacaattaatagactggatggaggcggataaagttgcaggaccacttctgcgctcggcccttccggctggctggtttattgctgataaatctggagccggtgagcgtgggtctcgcggtatcattgcagcactggggccagatggtaagccctcccgtatcgtagttatctacacgacggggagtcaggcaactatggatgaacgaaatagacagatcgctgagataggtgcctcactgattaagcattggtaactgtcagaccaagtttactcatatatactttagattgatttaaaacttcatttttaatttaaaaggatctaggtgaagatcctttttgataatctcatgaccaaaatcccttaacgtgagttttcgttccactgagcgtcagaccccgtagaaaagatcaaaggatcttcttgagatcctttttttctgcgcgtaatctgctgcttgcaaacaaaaaaaccaccgctaccagcggtggtttgtttgccggatcaagagctaccaactctttttccgaaggtaactggcttcagcagagcgcagataccaaatactgtccttctagtgtagccgtagttaggccaccacttcaagaactctgtagcaccgcctacatacctcgctctgctaatcctgttaccagtggctgctgccagtggcgataagtcgtgtcttaccgggttggactcaagacgatagttaccggataaggcgcagcggtcgggctgaacggggggttcgtgcacacagcccagcttggagcgaacgacctacaccgaactgagatacctacagcgtgagctatgagaaagcgccacgcttcccgaagggagaaaggcggacaggtatccggtaagcggcagggtcggaacaggagagcgcacgagggagcttccagggggaaacgcctggtatctttatagtcctgtcgggtttcgccacctctgacttgagcgtcgatttttgtgatgctcgtcaggggggcggagcctatggaaaaacgccagcaacgcggcctttttacggttcctggccttttgctggccttttgctcacatgttctttcctgcgttatcccctgattctgtggataaccgtattaccgcctttgagtgagctgataccgctcgccgcagccgaacgaccgagcgcagcgagtcagtgagcgaggaagcggaagagcgcccaatacgcaaaccgcctctccccgcgcgttggccgattcattaatg

SEQ ID NO: 9 - DNA, 8620 bp, Artificial Sequence
  Synthesized
cagcagctggcgtaatagcgaagaggcccgcaccgatcgcccttcccaacagttgcgcagcctgaatggcgaatggaattccagacgattgagcgtcaaaatgtaggtatttccatgagcgtttttcctgttgcaatggctggcggtaatattgttctggatattaccagcaaggccgatagtttgagttcttctactcaggcaagtgatgttattactaatcaaagaagtattgcgacaacggttaatttgcgtgatggacagactcttttactcggtggcctcactgattataaaaacacttctcaggattctggcgtaccgttcctgtctaaaatccctttaatcggcctcctgtttagctcccgctctgattctaacgaggaaagcacgttatacgtgctcgtcaaagcaaccatagtacgcgccctgtagcggcgcattaagcgcggcgggtgtggtggttacgcgcagcgtgaccgctacacttgccagcgccctagcgcccgctcctttcgctttcttcccttcctttctcgccacgttcgccggctttccccgtcaagctctaaatcgggggctccctttagggttccgatttagtgctttacggcacctcgaccccaaaaaacttgattagggtgatggttcacgtagtgggccatcgccctgatagacggtttttcgccctttgacgttggagtccacgttctttaatagtggactcttgttccaaactggaacaacactcaaccctatctcggtctattcttttgatttataagggattttgccgatttcggcctattggttaaaaaatgagctgatttaacaaaaatttaacgcgaattttaacaaaatattaacgtttacaatttaaatatttgcttatacaatcttcctgtttttggggcttttctgattatcaaccggggtacatatgattgacatgctagttttacgattaccgttcatcgccctgcgcgctcgctcgctcactgaggccgcccgggcaaagcccgggcgtcgggcgacctttggtcgcccggcctcagtgagcgagcgagcgcgcagagagggagtggaattcacgcgtgggcccctcaatattggccattagccatattattcattggttatatagcataaatcaatattggctattggccattgcatacgttgtatctatatcataatatgtacatttatattggctcatgtccaatatgaccgccatgttggcattgattattgactagttattaatagtaatcaattacggggtcattagttcatagcccatatatggagttccgcgttacataacttacggtaaatggcccgcctggctgaccgcccaacgacccccgcccattgacgtcaataatgacgtatgttcccatagtaacgccaatagggactttccattgacgtcaatgggtggagtatttacggtaaactgcccacttggcagtacatcaagtgtatcatatgccaagtccgccccctattgacgtcaatgacggtaaatggcccgcctggcattatgcccagtacatgaccttacgggactttcctacttggcagtacatctacgtattagtcatcgctattaccatgatgatgcggttttggcagtacaccaatgggcgtggatagcggtttgactcacggggatttccaagtctccaccccattgacgtcaatgggagtttgttttggcaccaaaatcaacgggactttccaaaatgtcgtaataaccccgccccgttgacgcaaatgggcggtaggcgtgtacggtgggaggtctatataagcagagctcgtttagtgaaccgtcagatcactagaagcttaattgtgagcgctcacaattgtgagactgctgccgcagtcagtaattgtgagcgctcacaattgacctggagctgcaggagttggtaattgtgagcgctcacaattcgtgaggcactgggcaggctagccaccatggcaccgaagaagaagcgcaaggtgcatatgaatacaaaatataataaggtaagtatcaaggttacaagacaggtttaaggcgccaatagaaacgggtgtggtacgcagccactggcttgtcgagacagagaagactcttgcgtttctgataggcacctattggtcttactgacatccactttgcctttctctccacaggagttcttactctacttagcagggtttgtagacggtgacggttccatctatgcccgtatctttaagggtcaacattggaagttcaagcactatattcgtttgaccttctgtgtgcggcagaagacacagcgccgttggttcctcgacaagctggtggacgagatcggtgtgggttacgtgactgactctggcagcgtttccgcttactatctgtccgagatcaagcctttgcataattttttaacacaactacaaccttttctaaaactaaaacaaaaacaagcaaatttagttttaaaaattattgaacaacttccgtcagcaaaagaatccccggacaaattcttagaagtttgtacatgggtggatcaaattgcagctctgaatgattcgaagacgcgtaaaacaacttctgaaaccgttcgtgctgtgctagacagtttaccaggatccgtgggaggtctatcgccatctcaggcatccagcgccgcatcctcggcttcctcaagcccgggttcagggatctccgaagcactcagagctggagcaggttccggcactggatacaacaaggaattcctgctctacctggcgggcttcgtcgacggggacggctccatctgggcctcgatcattcctgagcaaggttataagttcaagcacaggctgcgtctctctttcactgtcgctcagaagacacagcgccgttggttcctcgacaagctggtggacgagatcggtgtgggttacgtggttgaccagggcagcgtctccgagtacaggctgtccgagatcaagcctctgcacaacttcctgacccagctccagcccttcctgaagctcaagcagaagcaggccaacctcgtgctgaagatcatcgagcagctgccctccgccaaggaatccccggacaagttcctggaggtgtgcacctgggtggaccagatcgccgctctgaacgactccaagacccgcaagaccacttccgaaaccgtccgcgccgttctagacagtctctccgagaagaagaagtcgtccccctaagcggccgcgactctagatcataatcagccataccacatttgtagaggttttacttgctttaaaaaacctcccacacctccccctgaacctgaaacataaaatgaatgcaattgttgttgttaacttgtttattgcagcttataatggttacaaataaagcaatagcatcacaaatttcacaaataaagcatttttttcactgcattctagttgtggtttgtccaaactcatcaatgtatcttaaggcgggaattgatctaggaacccctagtgatggagttggccactccctctctgcgcgctcgctcgctcactgaggccgcccgggcaaagcccgggcgtcgggcgacctttggtcgcccggcctcagtgagcgagcgagcgcgcagagagggagtggccaaccccccccccccccccccggcgattctcttgtttgctccagactctcaggcaatgacctgatagcctttgtagagacctctcaaaaatagctaccctctccggcatgaatttatcagctagaacggttgaatatcatattgatggtgatttgactgtctccggcctttctcacccgtttgaatctttacctacacattactcaggcattgcatttaaaatatatgagggttctaaaaatttttatccttgcgttgaaataaaggcttctcccgcaaaagtattacagggtcataatgtttttggtacaaccgatttagctttatgctctgaggctttattgcttaattttgctaattctttgccttgcctgtatgatttattggatgttggaattcctgatgcggtattttctccttacgcatctgtgcggtatttcacaccgcatatggtgcactctcagtacaatctgctctgatgccgcatagttaagccagccccgacacccgccaacacccgctgacgcgccctgacgggcttgtctgctcccggcatccgcttacagacaagctgtgaccgtctccgggagctgcatgtgtcagaggttttcaccgtcatcaccgaaacgcgcgagacgaaagggcctcgtgatacgcctatttttataggttaatgtcatgataataatggtttcttagacgtcaggtggcacttttcggggaaatgtgcgcggaacccctatttgtttatttttctaaatacattcaaatatgtatccgctcatgagacaataaccctgataaatgcttcaataatattgaaaaaggaagagtatgagtattcaacatttccgtgtcgcccttattcccttttttgcggcattttgccttcctgtttttgctcacccagaaacgctggtgaaagtaaaagatgctgaagatcagttgggtgcacgagtgggttacatcgaactggatctcaacagcggtaagatccttgagagttttcgccccgaagaacgttttccaatgatgagcacttttaaagttctgctatgtggcgcggtattatcccgtattgacgccgggcaagagcaactcggtcgccgcatacactattctcagaatgacttggttgagtactcaccagtcacagaaaagcatcttacggatggcatgacagtaagagaattatgcagtgctgccataaccatgagtgataacactgcggccaacttacttctgacaacgatcggaggaccgaaggagctaaccgcttttttgcacaacatgggggatcatgtaactcgccttgatcgttgggaaccggagctgaatgaagccataccaaacgacgagcgtgacaccacgatgcctgtagcaatggcaacaacgttgcgcaaactattaactggcgaactacttactctagcttcccggcaacaattaatagactggatggaggcggataaagttgcaggaccacttctgcgctcggcccttccggctggctggtttattgctgataaatctggagccggtgagcgtgggtctcgcggtatcattgcagcactggggccagatggtaagccctcccgtatcgtagttatctacacgacggggagtcaggcaactatggatgaacgaaatagacagatcgctgagataggtgcctcactgattaagcattggtaactgtcagaccaagtttactcatatatactttagattgatttaaaacttcatttttaatttaaaaggatctaggtgaagatcctttttgataatctcatgaccaaaatcccttaacgtgagttttcgttccactgagcgtcagaccccgtagaaaagatcaaaggatcttcttgagatcctttttttctgcgcgtaatctgctgcttgcaaacaaaaaaaccaccgctaccagcggtggtttgtttgccggatcaagagctaccaactctttttccgaaggtaactggcttcagcagagcgcagataccaaatactgtccttctagtgtagccgtagttaggccaccacttcaagaactctgtagcaccgcctacatacctcgctctgctaatcctgttaccagtggctgctgccagtggcgataagtcgtgtcttaccgggttggactcaagacgatagttaccggataaggcgcagcggtcgggctgaacggggggttcgtgcacacagcccagcttggagcgaacgacctacaccgaactgagatacctacagcgtgagctatgagaaagcgccacgcttcccgaagggagaaaggcggacaggtatccggtaagcggcagggtcggaacaggagagcgcacgagggagcttccagggggaaacgcctggtatctttatagtcctgtcgggtttcgccacctctgacttgagcgtcgatttttgtgatgctcgtcaggggggcggagcctatggaaaaacgccagcaacgcggcctttttacggttcctggccttttgctggccttttgctcacatgtttattgcagcttataatggttacaaataaagcaatagcatcacaaatttcacaaataaagcatttttttcactgcattctagttgtggtttgtccaaactcatcaatgtatcttatcatgtctgctcgaagcggccgcggtacctcactgcccgctttccagtcgggaaacctgtcgtgccagctgcattaatgaatcggccaacgcgcggggagaggcggtttgcgtattgggcgccagggtggtttttcttttcaccagtgagacgggcaacagctgattgcccttcaccgcctggccctgagagagttgcagcaagcggtccacgctggtttgccccagcaggcgaaaatcctgtttgatggtggttaacggcgggatataacatgagctgtcttcggtatcgtcgtatcccactaccgagatatccgcaccaacgcgcagcccggactcggtaatggcgcgcattgcgcccagcgccatctgatcgttggcaaccagcatcgcagtgggaacgatgccctcattcagcatttgcatggtttgttgaaaaccggacatggcactccagtcgccttcccgttccgctatcggctgaatttgattgcgagtgagatatttatgccagccagccagacgcagacgcgccgagacagaacttaatgggcccgctaacagcgcgatttgctggtgacccaatgcgaccagatgctccacgcccagtcgcgtaccgtcttcatgggagaaaataatactgttgatgggtgtctggtcagagacatcaagaaataacgccggaacattagtgcaggcagcttccacagcaatggcatcctggtcatccagcggatagttaatgatcagcccactgacgcgttgcgcgagaagattgtgcaccgccgctttacaggcttcgacgccgcttcgttctaccatcgacaccaccacgctggcacccagttgatcggcgcgagatttaatcgccgcgacaatttgcgacggcgcgtgcagggccagactggaggtggcaacgccaatcagcaacgactgtttgcccgccagttgttgtgccacgcggttgggaatgtaattcagctccgccatcgccgcttccactttttcccgcgttttcgcagaaacgtggctggcctggttcaccacgcgggaaacggtctgataagagacaccggcatactctgcgacatcgtataacgttactggtttcaccatggtggctcgagctatagtgagtcgtattaagtactctagccttaagagctgtaattgaactgggagtggacacctgtggagagaaaggcaaagtggatgtcagtaagaccaataggtgcctatcagaaacgcaagagtcttctctgtctcgacaagcccagtttctattggtctccttaaacctgtcttgtaaccttgatacttacctgcccagtgcctcacgaccaacttctgcagcttaagttcgagactgttgtgtcagaagcactgactgcgttagcaatttaactgtgataaactaccgcaataaagcttctagtgatctgacggttcactaaacgagctctgcttatatagacctcccaccgtacacgcctaccgcccatttgcgtcaacggggcggggttattacgacattttggaaagtcccgttgattttggtgccaaaacaaactcccattgacgtcaatggggtggagacttggaaatccccgtgagtcaaaccgctatccacgcccattggtgtactgccaaaaccgcatcaccatggtaatagcgatgactaatacgtagatgtactgccaagtaggaaagtcccgtaaggtcatgtactgggcataatgccaggcgggccatttaccgtcattgacgtcaatagggggcggacttggcatatgatacacttgatgtactgccaagtgggcagtttaccgtaaatactccacccattgacgtcaatggaaagtccctattggcgttactatgggaacatacgtcattattgacgtcaatgggcgggggtcgttgggcggtcagccaggcgggccatttaccgtaagttatgtaacgcggaactccatatatgggctatgaactaatgaccccgtaattgattactattaataactagtcaataatcaatgccaacatggcggtcatattggacatgagccaatataaatgtacatattatgatatagatacaacgtatgcaatggccaatagccaatattgatttatgctatataaccaatgaataatatggctaatggccaatattgaacatgttctttcctgcgttatcccctgattctgtggataaccgtattaccgcctttgagtgagctgataccgctcgccgcagccgaacgaccgagcgcagcgagtcagtgagcgaggaagcggaagagcgcccaatacgcaaaccgcctctccccgcgcgttggccgattcattaatg

SEQ ID NO: 10 - DNA, 6609 bp, Artificial Sequence
  Synthesized
cagcagctggcgtaatagcgaagaggcccgcaccgatcgcccttcccaacagttgcgcagcctgaatggcgaatggaattccagacgattgagcgtcaaaatgtaggtatttccatgagcgtttttcctgttgcaatggctggcggtaatattgttctggatattaccagcaaggccgatagtttgagttcttctactcaggcaagtgatgttattactaatcaaagaagtattgcgacaacggttaatttgcgtgatggacagactcttttactcggtggcctcactgattataaaaacacttctcaggattctggcgtaccgttcctgtctaaaatccctttaatcggcctcctgtttagctcccgctctgattctaacgaggaaagcacgttatacgtgctcgtcaaagcaaccatagtacgcgccctgtagcggcgcattaagcgcggcgggtgtggtggttacgcgcagcgtgaccgctacacttgccagcgccctagcgcccgctcctttcgctttcttcccttcctttctcgccacgttcgccggctttccccgtcaagctctaaatcgggggctccctttagggttccgatttagtgctttacggcacctcgaccccaaaaaacttgattagggtgatggttcacgtagtgggccatcgccctgatagacggtttttcgccctttgacgttggagtccacgttctttaatagtggactcttgttccaaactggaacaacactcaaccctatctcggtctattcttttgatttataagggattttgccgatttcggcctattggttaaaaaatgagctgatttaacaaaaatttaacgcgaattttaacaaaatattaacgtttacaatttaaatatttgcttatacaatcttcctgtttttggggcttttctgattatcaaccggggtacatatgattgacatgctagttttacgattaccgttcatcgccctgcgcgctcgctcgctcactgaggccgcccgggcaaagcccgggcgtcgggcgacctttggtcgcccggcctcagtgagcgagcgagcgcgcagagagggagtggaattcacgcgtgggcccctcaatattggccattagccatattattcattggttatatagcataaatcaatattggctattggccattgcatacgttgtatctatatcataatatgtacatttatattggctcatgtccaatatgaccgccatgttggcattgattattgactagttattaatagtaatcaattacggggtcattagttcatagcccatatatggagttccgcgttacataacttacggtaaatggcccgcctggctgaccgcccaacgacccccgcccattgacgtcaataatgacgtatgttcccatagtaacgccaatagggactttccattgacgtcaatgggtggagtatttacggtaaactgcccacttggcagtacatcaagtgtatcatatgccaagtccgccccctattgacgtcaatgacggtaaatggcccgcctggcattatgcccagtacatgaccttacgggactttcctacttggcagtacatctacgtattagtcatcgctattaccatgatgatgcggttttggcagtacaccaatgggcgtggatagcggtttgactcacggggatttccaagtctccaccccattgacgtcaatgggagtttgttttggcaccaaaatcaacgggactttccaaaatgtcgtaataaccccgccccgttgacgcaaatgggcggtaggcgtgtacggtgggaggtctatataagcagagctcgtttagtgaaccgtcagatcactagaagcttaattgtgagcgctcacaattgtgagactgctgccgcagtcagtaattgtgagcgctcacaattgacctggagctgcaggagttggtaattgtgagcgctcacaattcgtgaggcactgggcaggctagccaccatggcaccgaagaagaagcgcaaggtgcatatgaatacaaaatataataaggtaagtatcaaggttacaagacaggtttaaggcgccaatagaaacgggtgtggtacgcagccactggcttgtcgagacagagaagactcttgcgtttctgataggcacctattggtcttactgacatccactttgcctttctctccacaggagttcttactctacttagcagggtttgtagacggtgacggttccatctatgcccgtatctttaagggtcaacattggaagttcaagcactatattcgtttgaccttctgtgtgcggcagaagacacagcgccgttggttcctcgacaagctggtggacgagatcggtgtgggttacgtgactgactctggcagcgtttccgcttactatctgtccgagatcaagcctttgcataattttttaacacaactacaaccttttctaaaactaaaacaaaaacaagcaaatttagttttaaaaattattgaacaacttccgtcagcaaaagaatccccggacaaattcttagaagtttgtacatgggtggatcaaattgcagctctgaatgattcgaagacgcgtaaaacaacttctgaaaccgttcgtgctgtgctagacagtttaccaggatccgtgggaggtctatcgccatctcaggcatccagcgccgcatcctcggcttcctcaagcccgggttcagggatctccgaagcactcagagctggagcaggttccggcactggatacaacaaggaattcctgctctacctggcgggcttcgtcgacggggacggctccatctgggcctcgatcattcctgagcaaggttataagttcaagcacaggctgcgtctctctttcactgtcgctcagaagacacagcgccgttggttcctcgacaagctggtggacgagatcggtgtgggttacgtggttgaccagggcagcgtctccgagtacaggctgtccgagatcaagcctctgcacaacttcctgacccagctccagcccttcctgaagctcaagcagaagcaggccaacctcgtgctgaagatcatcgagcagctgccctccgccaaggaatccccggacaagttcctggaggtgtgcacctgggtggaccagatcgccgctctgaacgactccaagacccgcaagaccacttccgaaaccgtccgcgccgttctagacagtctctccgagaagaagaagtcgtccccctaagcggccgcgactctagatcataatcagccataccacatttgtagaggttttacttgctttaaaaaacctcccacacctccccctgaacctgaaacataaaatgaatgcaattgttgttgttaacttgtttattgcagcttataatggttacaaataaagcaatagcatcacaaatttcacaaataaagcatttttttcactgcattctagttgtggtttgtccaaactcatcaatgtatcttaaggcgggaattgatctaggaacccctagtgatggagttggccactccctctctgcgcgctcgctcgctcactgaggccgcccgggcaaagcccgggcgtcgggcgacctttggtcgcccggcctcagtgagcgagcgagcgcgcagagagggagtggccaaccccccccccccccccccggcgattctcttgtttgctccagactctcaggcaatgacctgatagcctttgtagagacctctcaaaaatagctaccctctccggcatgaatttatcagctagaacggttgaatatcatattgatggtgatttgactgtctccggcctttctcacccgtttgaatctttacctacacattactcaggcattgcatttaaaatatatgagggttctaaaaatttttatccttgcgttgaaataaaggcttctcccgcaaaagtattacagggtcataatgtttttggtacaaccgatttagctttatgctctgaggctttattgcttaattttgctaattctttgccttgcctgtatgatttattggatgttggaattcctgatgcggtattttctccttacgcatctgtgcggtatttcacaccgcatatggtgcactctcagtacaatctgctctgatgccgcatagttaagccagccccgacacccgccaacacccgctgacgcgccctgacgggcttgtctgctcccggcatccgcttacagacaagctgtgaccgtctccgggagctgcatgtgtcagaggttttcaccgtcatcaccgaaacgcgcgagacgaaagggcctcgtgatacgcctatttttataggttaatgtcatgataataatggtttcttagacgtcaggtggcacttttcggggaaatgtgcgcggaacccctatttgtttatttttctaaatacattcaaatatgtatccgctcatgagacaataaccctgataaatgcttcaataatattgaaaaaggaagagtatgagtattcaacatttccgtgtcgcccttattcccttttttgcggcattttgccttcctgtttttgctcacccagaaacgctggtgaaagtaaaagatgctgaagatcagttgggtgcacgagtgggttacatcgaactggatctcaacagcggtaagatccttgagagttttcgccccgaagaacgttttccaatgatgagcacttttaaagttctgctatgtggcgcggtattatcccgtattgacgccgggcaagagcaactcggtcgccgcatacactattctcagaatgacttggttgagtactcaccagtcacagaaaagcatcttacggatggcatgacagtaagagaattatgcagtgctgccataaccatgagtgataacactgcggccaacttacttctgacaacgatcggaggaccgaaggagctaaccgcttttttgcacaacatgggggatcatgtaactcgccttgatcgttgggaaccggagctgaatgaagccataccaaacgacgagcgtgacaccacgatgcctgtagcaatggcaacaacgttgcgcaaactattaactggcgaactacttactctagcttcccggcaacaattaatagactggatggaggcggataaagttgcaggaccacttctgcgctcggcccttccggctggctggtttattgctgataaatctggagccggtgagcgtgggtctcgcggtatcattgcagcactggggccagatggtaagccctcccgtatcgtagttatctacacgacggggagtcaggcaactatggatgaacgaaatagacagatcgctgagataggtgcctcactgattaagcattggtaactgtcagaccaagtttactcatatatactttagattgatttaaaacttcatttttaatttaaaaggatctaggtgaagatcctttttgataatctcatgaccaaaatcccttaacgtgagttttcgttccactgagcgtcagaccccgtagaaaagatcaaaggatcttcttgagatcctttttttctgcgcgtaatctgctgcttgcaaacaaaaaaaccaccgctaccagcggtggtttgtttgccggatcaagagctaccaactctttttccgaaggtaactggcttcagcagagcgcagataccaaatactgtccttctagtgtagccgtagttaggccaccacttcaagaactctgtagcaccgcctacatacctcgctctgctaatcctgttaccagtggctgctgccagtggcgataagtcgtgtcttaccgggttggactcaagacgatagttaccggataaggcgcagcggtcgggctgaacggggggttcgtgcacacagcccagcttggagcgaacgacctacaccgaactgagatacctacagcgtgagctatgagaaagcgccacgcttcccgaagggagaaaggcggacaggtatccggtaagcggcagggtcggaacaggagagcgcacgagggagcttccagggggaaacgcctggtatctttatagtcctgtcgggtttcgccacctctgacttgagcgtcgatttttgtgatgctcgtcaggggggcggagcctatggaaaaacgccagcaacgcggcctttttacggttcctggccttttgctggccttttgctcacatgtttattgcagcttataatggttacaaataaagcaatagcatcacaaatttcacaaataaagcatttttttcactgcattctagttgtggtttgtccaaactcatcaatgtatcttatcatgtctgctcgaagcggccgcggtaccaacatggcggtcatattggacatgagccaatataaatgtacatattatgatatagatacaacgtatgcaatggccaatagccaatattgatttatgctatataaccaatgaataatatggctaatggccaatattgaacatgttctttcctgcgttatcccctgattctgtggataaccgtattaccgcctttgagtgagctgataccgctcgccgcagccgaacgaccgagcgcagcgagtcagtgagcgaggaagcggaagagcgcccaatacgcaaaccgcctctccccgcgcgttggccgattcattaatg